European Patent Specification EP 3 886 987 B1, published November 15, 2023. Title: Compounds Useful in HIV Therapy. Applicant: GlaxoSmithKline Intellectual Property Development Limited The University of North Carolina at Chapel Hill ViiV Healthcare Company De La Rosa, Martha Tai, Vincent Tang, Jun Dunham, Richard Margolis, David. The sequence listing filed with the application follows.

SEQUENCE LISTING (4 sequences)

SEQ ID NO: 1 - DNA, 22 bp, synthetic primer
atcaagcagctatgcaaatgtt

SEQ ID NO: 2 - DNA, 30 bp, synthetic primer
ctgaagggtactagtagttcctgctatgtc

SEQ ID NO: 3 - DNA, 29 bp, synthetic probe
accatcaatgaggaagctgcagaatggga

SEQ ID NO: 4 - DNA, 152 bp, Synthetic standard control
atcaagcagccatgcaaatgttaaaagagaccatcaatgaggaagctgcagaatgggatagattgcatccagtgcatgcagggcctattgcaccaggccagatgagagaaccaaggggaagtgacatagcaggaactactagtacccttcag